European Patent Application EP 4 763 209 A1, published June 24, 2026. Title: USE OF αS-SETMAR AGONIST FOR PREVENTING OR TREATING GLIOBLASTOMA. Applicant: INSERM (Institut National de la Sante et de la Recherche Medicale). The sequence listing filed with the application follows.

SEQUENCE LISTING (4 sequences)

SEQ ID NO: 1 - DNA, 2055 bp, Homo sapiens
  source 1..2055: mol_type = genomic DNA
atgttcgcggaagcggcaaagacgacacggccttgtgggatggcggagtttaaggagaagcctgaggccccgactgagcagctggatgtcgcgtgcggccaggaaaacttgccggtgggcgcgtggcccccgggggccgcgccggcgcccttccagtacactcctgatcatgtagttggacctggagcagacattgatcccactcaaataacctttcccggatgcatttgtgtcaaaactccctgcctccctggcacttgctcctgtctccgccatggagagaactatgatgataactcatgccttagagatataggatctggaggaaagtatgcagagcctgtttttgaatgcaatgtcctgtgccgatgcagtgaccactgcagaaacagagtggtccagaaaggtctacagttccacttccaagtgttcaagacgcataaaaaaggctggggacttcgtaccttggaatttataccgaaaggaaggtttgtctgtgaatatgctggtgaggttttaggattctctgaagttcagagaagaattcacttacaaacaaaatccgactccaattacattatagccatcagggaacatgtttataatgggcaggtaatggaaacatttgttgaccctacttatataggaaatattggaagattccttaatcattcttgtgagccaaaccttttgatgattcctgtccgaattgactcaatggtacctaagttggcactttttgcagccaaagatattgtgccagaagaagaactctcttatgattattcaggaagatatcttaatctaacagtcagtgaagacaaagaaaggctagatcatgggaaactaaggaaaccttgttactgtggtgccaaatcatgtactgctttcctgccttttgacagttctctgtactgccccgtagaaaagtcgaacatcagttgtggaaatgagaaggaacccagcatgtgtggctcagccccttctgtgttcccctcctgcaagcgattgacccttgagactatgaaaatgatgttagacaaaaagcaaattcgagcaattttcttattcgagttcaaaatgggtcgtaaagcagcagaaacaactcgcaacatcaacaatgcatttggcccaggaactgctaacgaacgtacagtgcagtggtggttcaagaagttttgcaaaggagatgagagccttgaagatgaggagcgtagtggccggccatcagaagttgacaacgaccagttgagagcaatcatcgaagctgatccccttacaactacacgagaagttgctgaagaactcaatgtcaaccattctacggtcgttcgacatttgaagcaaattggaaaggtgaaaaagctcgataagtgggtgcctcatgagctgactgaaaatcaaaaaaatcgtcgttttgaagtgtcatcttctcttattctacgcaaccacaacgaaccatttctcgatcggattgtgacgtgtgatgaaaagtggattttatatgacaaccggcgacgatcagctcagtggttggatcaagaagaagctccaaagcacttcccaaagccaatcttgcacccaaaaaaggtcatggtcactatttggtggtctgctgctggtctgatccactacagctttctgaatcccggtgaaaccattacatctgagaagtatgctcaggaaatcgatgagatgaaccaaaaactgcaacgcctgcagctggcattggtcaacagaaagggcccaattcttctccacgacaatgcccgaccgcatgttgcacaacccacacttcaaaagttgaatgaattgggctatgaagttttgcctcatccaccgtattcacctgacctcttgccaaccaactaccacgtctttaagcatctcaacaactttttgcagggaaaacgcttccacaaccagcaggatgcagaaaatgctttccaagagttcgtcgaatcccaaagcacggatttttacgctacaggaataaaccaacttatttctcgttggcaaaaatgtgttgattgtaatggttcctattttgattaa

SEQ ID NO: 2 - protein, 684 aa, Homo sapiens
MFAEAAKTTRPCGMAEFKEKPEAPTEQLDVACGQENLPVGAWPPGAAPAPFQYTPDHVVGPGADIDPTQITFPGCICVKTPCLPGTCSCLRHGENYDDNSCLRDIGSGGKYAEPVFECNVLCRCSDHCRNRVVQKGLQFHFQVFKTHKKGWGLRTLEFIPKGRFVCEYAGEVLGFSEVQRRIHLQTKSDSNYIIAIREHVYNGQVMETFVDPTYIGNIGRFLNHSCEPNLLMIPVRIDSMVPKLALFAAKDIVPEEELSYDYSGRYLNLTVSEDKERLDHGKLRKPCYCGAKSCTAFLPFDSSLYCPVEKSNISCGNEKEPSMCGSAPSVFPSCKRLTLETMKMMLDKKQIRAIFLFEFKMGRKAAETTRNINNAFGPGTANERTVQWWFKKFCKGDESLEDEERSGRPSEVDNDQLRAIIEADPLTTTREVAEELNVNHSTVVRHLKQIGKVKKLDKWVPHELTENQKNRRFEVSSSLILRNHNEPFLDRIVTCDEKWILYDNRRRSAQWLDQEEAPKHFPKPILHPKKVMVTIWWSAAGLIHYSFLNPGETITSEKYAQEIDEMNQKLQRLQLALVNRKGPILLHDNARPHVAQPTLQKLNELGYEVLPHPPYSPDLLPTNYHVFKHLNNFLQGKRFHNQQDAENAFQEFVESQSTDFYATGINQLISRWQKCVDCNGSYFD

SEQ ID NO: 3 - DNA, 1191 bp, Homo sapiens
  source 1..1191: mol_type = genomic DNA
atgttcgcggaagcggcaaagacgacacggccttgtgggatggcggagtttaaggagaagcctgaggccccgactgagcagctggatgtcgcgtgcggccaggaaaacttgccggtgggcgcgtggcccccgggggccgcgccggcgcccttccagactatgaaaatgatgttagacaaaaagcaaattcgagcaattttcttattcgagttcaaaatgggtcgtaaagcagcagaaacaactcgcaacatcaacaatgcatttggcccaggaactgctaacgaacgtacagtgcagtggtggttcaagaagttttgcaaaggagatgagagccttgaagatgaggagcgtagtggccggccatcagaagttgacaacgaccagttgagagcaatcatcgaagctgatccccttacaactacacgagaagttgctgaagaactcaatgtcaaccattctacggtcgttcgacatttgaagcaaattggaaaggtgaaaaagctcgataagtgggtgcctcatgagctgactgaaaatcaaaaaaatcgtcgttttgaagtgtcatcttctcttattctacgcaaccacaacgaaccatttctcgatcggattgtgacgtgtgatgaaaagtggattttatatgacaaccggcgacgatcagctcagtggttggatcaagaagaagctccaaagcacttcccaaagccaatcttgcacccaaaaaaggtcatggtcactatttggtggtctgctgctggtctgatccactacagctttctgaatcccggtgaaaccattacatctgagaagtatgctcaggaaatcgatgagatgaaccaaaaactgcaacgcctgcagctggcattggtcaacagaaagggcccaattcttctccacgacaatgcccgaccgcatgttgcacaacccacacttcaaaagttgaatgaattgggctatgaagttttgcctcatccaccgtattcacctgacctcttgccaaccaactaccacgtctttaagcatctcaacaactttttgcagggaaaacgcttccacaaccagcaggatgcagaaaatgctttccaagagttcgtcgaatcccaaagcacggatttttacgctacaggaataaaccaacttatttctcgttggcaaaaatgtgttgattgtaatggttcctattttgattaa

SEQ ID NO: 4 - protein, 396 aa, Homo sapiens
MFAEAAKTTRPCGMAEFKEKPEAPTEQLDVACGQENLPVGAWPPGAAPAPFQTMKMMLDKKQIRAIFLFEFKMGRKAAETTRNINNAFGPGTANERTVQWWFKKFCKGDESLEDEERSGRPSEVDNDQLRAIIEADPLTTTREVAEELNVNHSTVVRHLKQIGKVKKLDKWVPHELTENQKNRRFEVSSSLILRNHNEPFLDRIVTCDEKWILYDNRRRSAQWLDQEEAPKHFPKPILHPKKVMVTIWWSAAGLIHYSFLNPGETITSEKYAQEIDEMNQKLQRLQLALVNRKGPILLHDNARPHVAQPTLQKLNELGYEVLPHPPYSPDLLPTNYHVFKHLNNFLQGKRFHNQQDAENAFQEFVESQSTDFYATGINQLISRWQKCVDCNGSYFD